European Patent Application EP 4 349 329 A1, published April 10, 2024. Title: A benzyloxybenzylaminyl amino acid derivative for modulating TSLP/TSLPR signaling. Applicant: AMTIXBIO. CO. LTD. The sequence listing filed with the application follows.

SEQUENCE LISTING (6 sequences)

SEQ ID NO: 1 - DNA, 1113 bp, Artificial Sequence
  mouse TSLPR, CDS
atggcatgggcactcgcggtcatcctcctgcctcggctccttgcggcggcagcggcggcggcggcggtgacgtcacggggtgatgtcacagtcgtctgccatgacctggagacggtggaggtcacgtggggctcgggccccgaccaccacggcgccaacttgagcctggagttccgttatggcactggcgccctgcaaccctgcccgcgatatttcctgtccggcgctggtgtcacttccgggtgcatcctccccgcggcgagggcggggctgctggagctggcactgcgcgacggaggcggggccatggtgtttaaggctaggcagcgcgcgtccgcctggctgaagccccgcccaccttggaatgtgacgctgctctggacaccagacggggacgtgactgtctcctggcctgcccactcctacctgggcctggactacgaggtgcagcaccgggagagcaatgacgatgaggacgcctggcagacgacctcagggccctgctgtgacttgacagtgggcgggctcgaccccgtacgctgctatgacttccgggttcgggcgtcgccccgggccgcgcactatggcctggaggcgcagcctagcgagtggacagcggtgacaaggctttccggggcagcatccgcgggtgacccctgcgccgcccaccttccccccctagcctcctgtaccgcaagccccgccccatccccggccctggccccgcccctcctgcccctgggctgcggcctagcagcgctgctgacactgtccctgctcctggccgccctgaggcttcgcagggtgaaagatgcgctgctgccctgcgtccctgaccccagcggctccttccctggactctttgagaagcatcacgggaacttccaggcctggattgcggacgcccaggccacagccccgccagccaggaccgaggaggaagatgacctcatccacaccaaggctaagagggtggagcccgaggacggcacctccctctgcaccgtgccaaggccacccagcttcgagccaagggggccgggaggcggggccatggtgtcagtgggcggggccacgttcatggtgggcgacagcggctacatgaccctgtga

SEQ ID NO: 2 - DNA, 1116 bp, Artificial Sequence
  humas TSLPR, CDS
atggggcggctggttctgctgtggggagctgccgtctttctgctgggaggctggatggctttggggcaaggaggagcagcagaaggagtacagattcagatcatctacttcaatttagaaaccgtgcaggtgacatggaatgccagcaaatactccaggaccaacctgactttccactacagattcaacggtgatgaggcctatgaccagtgcaccaactaccttctccaggaaggtcacacttcggggtgcctcctagacgcagagcagcgagacgacattctctatttctccatcaggaatgggacgcaccccgttttcaccgcaagtcgctggatggtttattacctgaaacccagttccccgaagcacgtgagattttcgtggcatcaggatgcagtgacggtgacgtgttctgacctgtcctacggggatctcctctatgaggttcagtaccggagccccttcgacaccgagtggcagtccaaacaggaaaatacctgcaacgtcaccatagaaggcttggatgccgagaagtgttactctttctgggtcagggtgaaggctatggaggatgtatatgggccagacacatacccaagcgactggtcagaggtgacatgctggcagagaggcgagattcgggatgcctgtgcagagacaccaacgcctcccaaaccaaagctgtccaaatttattttaatttccagcctggccatccttctgatggtgtctctcctccttctgtctttatggaaattatggagagtgaagaagtttctcattcccagcgtgccagacccgaaatccatcttccccgggctctttgagatacaccaagggaacttccaggagtggatcacagacacccagaacgtggcccacctccacaagatggcaggtgcagagcaagaaagtggccccgaggagcccctggtagtccagttggccaagactgaagccgagtctcccaggatgctggacccacagaccgaggagaaagaggcctctgggggatccctccagcttccccaccagcccctccaaggcggtgatgtggtcacaatcgggggcttcacctttgtgatgaatgaccgctcctacgtggcgttgtga

SEQ ID NO: 3 - DNA, 1380 bp, Artificial Sequence
  mouse IL7R-alpha, CDS
atgatggctctgggtagagctttcgctatagttttctgcttaattcaagctgtttctggagaaagtggaaatgcccaggatggagacctagaagatgcagacgcggacgatcactccttctggtgccacagccagttggaagtggatggaagtcaacatttattgacttgtgcttttaatgactcagacatcaacacagctaatctggaatttcaaatatgtggggctcttttacgagtgaaatgcctaactcttaacaagctgcaagatatatattttataaagacatcagaattcttactgattggtagcagcaatatatgtgtgaagcttggacaaaagaatttaacttgcaaaaatatggctataaacacaatagttaaagccgaggctccctctgacctgaaagtcgtttatcgcaaagaagcaaatgattttttggtgacatttaatgcacctcacttgaaaaagaaatatttaaaaaaagtaaagcatgatgtggcctaccgcccagcaaggggtgaaagcaactggacgcatgtatctttattccacacaagaacaacaatcccacagagaaaactacgaccaaaagcaatgtatgaaatcaaagtccgatccattccccataacgattacttcaaaggcttctggagcgagtggagtccaagttctaccttcgaaactccagaacccaagaatcaaggaggatgggatcctgtcttgccaagtgtcaccattctgagtttgttctctgtgtttttgttggtcatcttagcccatgtgctatggaaaaaaaggattaaacctgtcgtatggcctagtctccccgatcataagaaaactctggaacaactatgtaagaagccaaaaacgagtctgaatgtgagtttcaatcccgaaagtttcctggactgccagattcatgaggtgaaaggcgttgaagccagggacgaggtggaaagttttctgcccaatgatcttcctgcacagccagaggagttggagacacagggacacagagccgctgtacacagtgcaaaccgctcgcctgagacttcagtcagcccaccagaaacagttagaagagagtcacccttaagatgcctggctagaaatctgagtacctgcaatgcccctccactcctttcctctaggtcccctgactacagagatggtgacagaaataggcctcctgtgtatcaagacttgctgccaaactctggaaacacaaatgtccctgtccctgtccctcaaccattgcctttccagtcgggaatcctgataccagtttctcagagacagcccatctccacttcctcagtactgaatcaagaagaagcgtatgtcaccatgtctagtttttaccaaaacaaatga

SEQ ID NO: 4 - DNA, 1380 bp, Artificial Sequence
  human IL7R-alpha, CDS
atgacaattctaggtacaacttttggcatggttttttctttacttcaagtcgtttctggagaaagtggctatgctcaaaatggagacttggaagatgcagaactggatgactactcattctcatgctatagccagttggaagtgaatggatcgcagcactcactgacctgtgcttttgaggacccagatgtcaacatcaccaatctggaatttgaaatatgtggggccctcgtggaggtaaagtgcctgaatttcaggaaactacaagagatatatttcatcgagacaaagaaattcttactgattggaaagagcaatatatgtgtgaaggttggagaaaagagtctaacctgcaaaaaaatagacctaaccactatagttaaacctgaggctccttttgacctgagtgtcgtctatcgggaaggagccaatgactttgtggtgacatttaatacatcacacttgcaaaagaagtatgtaaaagttttaatgcacgatgtagcttaccgccaggaaaaggatgaaaacaaatggacgcatgtgaatttatccagcacaaagctgacactcctgcagagaaagctccaaccggcagcaatgtatgagattaaagttcgatccatccctgatcactattttaaaggcttctggagtgaatggagtccaagttattacttcagaactccagagatcaataatagctcaggggagatggatcctatcttactaaccatcagcattttgagttttttctctgtcgctctgttggtcatcttggcctgtgtgttatggaaaaaaaggattaagcctatcgtatggcccagtctccccgatcataagaagactctggaacatctttgtaagaaaccaagaaaaaatttaaatgtgagtttcaatcctgaaagtttcctggactgccagattcatagggtggatgacattcaagctagagatgaagtggaaggttttctgcaagatacgtttcctcagcaactagaagaatctgagaagcagaggcttggaggggatgtgcagagccccaactgcccatctgaggatgtagtcatcactccagaaagctttggaagagattcatccctcacatgcctggctgggaatgtcagtgcatgtgacgcccctattctctcctcttccaggtccctagactgcagggagagtggcaagaatgggcctcatgtgtaccaggacctcctgcttagccttgggactacaaacagcacgctgccccctccattttctctccaatctggaatcctgacattgaacccagttgctcagggtcagcccattcttacttccctgggatcaaatcaagaagaagcatatgtcaccatgtccagcttctaccaaaaccagtga

SEQ ID NO: 5 - DNA, 3288 bp, Artificial Sequence
  mouse TRPA1, CDS
atgaagcgcggcttgaggaggattctgctcccggaggaaaggaaggaggtccagggcgttgtctatcgcggcgtcggggaagacatggactgctccaaggaatcctttaaggtggacattgaaggagatatgtgtagattagaagacttcatcaagaaccgaagaaaactaagcaaatatgaggatgaaaatctctgtcctctgcatcacgcagcagcagaaggtcaagttgaactgatggaactgatcatcaatggttcttcgtgtgaagtgctgaatataatggatggttatggaaataccccactgcattgtgctgcagaaaaaaatcaagttgaaagtgtaaagtttcttctcagccaaggagcaaatccaaacctccgaaatagaaacatgatgtcaccccttcacatagctgtgcatggcatgtacaacgaagtgatcaaggtgttgactgagcacaaggccactaacatcaatttagaaggagagaatgggaacacggctttgatgtccacgtgtgccaaagacaacagtgaagctttgcaaattttgttagaaaaaggagctaagctgtgtaaatcaaataagtggggagactaccctgtgcaccaggcagcattttcaggtgccaaaaaatgcatggaattaatcttagcatatggtgaaaagaacggctacagcagggagactcacattaattttgtgaatcacaagaaagccagccctctccacctagcagttcaaagcggagacttggacatgattaagatgtgcctggacaacggtgcacacatcgacatgatggagaatgccaaatgcatggccctccattttgctgcaacccagggagccactgacatcgttaagctcatgatctcatcctataccggaagtagtgatattgtgaatgcagttgatggcaatcaggagaccctgcttcacagagcctcgttatttgatcaccatgacctggcagaatacctaatatcagtgggagcagacatcaacagcactgattctgaaggacgctctccacttattttagcaacagcttctgcatcctggaacattgtgaatttgctcctctgtaaaggtgccaaagtagacataaaagatcatcttggacgtaactttttgcatttgactgtgcagcagccttatggactaagaaatttgcggcctgagtttatgcagatgcaacacatcaaagagctggtgatggatgaagacaatgacggatgcacacctctccattatgcctgtaggcagggggttcctgtctctgtaaataacctccttggcttcaatgtgtccattcatagcaaaagtaaagataagaagtcgcccctgcattttgcagccagttatgggcgcatcaatacatgtcagagacttctgcaagacataagtgatacgaggcttttgaatgaaggggatctccatgggatgacccctctccacctggcagcaaaaaatgggcatgataaagtcgttcaactccttctgaagaaaggggccttatttctcagtgaccacaatggctggactgctttgcatcacgcctccatgggtgggtacactcagaccatgaaggtcattcttgatactaacttgaaatgcacagaccgactagatgaagaagggaacacagcactccactttgcagcacgggaaggccatgccaaggctgttgcaatgcttttgagctacaatgctgacatcctcctgaacaagaagcaagcttcctttctgcatattgccctgcacaataagcgcaaggaagtggttctcacaaccatcagaaataaaagatgggatgagtgtcttcaagttttcactcataattctccaagcaatcgatgtccaatcatggagatggtagaatacctccccgagtgcatgaaagttcttttagatttctgcatgataccttccacagaagacaagtcctgtcaagactaccatattgagtataatttcaagtatctccaatgcccattatccatgaccaaaaaagtagcacctacccaggatgtggtatatgagcctcttacaatcctcaatgtcatggtccaacataaccgcatagaactcctcaaccaccctgtgtgtagggagtacttactcatgaaatggtgtgcctatggattcagagcccatatgatgaacctaggatcttattgtcttggtctcatacccatgacccttcttgttgtcaaaatacagcctggaatggccttcaattctactggaataatcaatggaactagtagtactcatgaggaaagaatagacactctgaaaaggaattacttcctggattacaacaatgctctggaatgggttatctatacaactagtatcatcttcgtgttgcccttgttcctcaacatcccagcgtatatgcagtggcaatgtggagcaatagcgatattcttctactggatgaacttcctactgtatcttcaaaggtttgagaactgtggaattttcattgttatgttggaggtgatttttaaaacattgctgagatcgaccggagtgtttatcttcctcctactggcttttggcctcagcttttatgttctcctgaatttccaagatgccttcagcaccccattgctttccttaatccagacattcagtatgatgctaggagacatcaattatcgagatgccttcctagaaccattgtttagaaatgagttggcatacccagtcctgacctttgggcagcttattgccttcacaatgtttgtcccaattgttctcatgaacttactgattggcttggcggttggggacattgctgaggtccagaagcatgcgtcattgaagaggattgctatgcaggtggaacttcataccaacttagaaaaaaagctgccactctggtacttacgcaaagtggatcagaggtccaccatcgtgtatccaaatagacccaggcacggcaggatgctacggttttttcattactttcttaatatgcaagaaacacgacaagaagtaccaaacattgacacatgcttggaaatggaaatattgaaacagaaatatcggctgaaggacctcacttccctcttggaaaagcagcatgagctcatcaaactcatcatccagaagatggagatcatctcagagacagaagatgaagataaccattgctctttccaagacaggttcaagaaggagaggctggaacagatgcacagcaagtggaattttgtcttaaacgcagttaagactaaaacacattgttctattagccacccggacttttag

SEQ ID NO: 6 - DNA, 3360 bp, Artificial Sequence
  human TRPA1, CDS
atgaagcgcagcctgaggaagatgtggcgccctggagaaaagaaggagccccagggcgttgtctatgaggatgtgccggacgacacggaggatttcaaggaatcgcttaaggtggtttttgaaggaagtgcatatggattacaaaactttaataagcaaaagaaattaaaaagatgtgacgatatggacaccttcttcttgcattatgctgcagcagaaggccaaattgagctaatggagaagatcaccagagattcctctttggaagtgctgcatgaaatggatgattatggaaatacccctctgcattgtgctgtagaaaaaaaccaaattgaaagcgttaagtttcttctcagcagaggagcaaacccaaatctccgaaacttcaacatgatggctcctctccacatagctgtgcagggcatgaataatgaggtgatgaaggtcttgcttgagcatagaactattgatgttaatttggaaggagaaaatggaaacacagctgtgatcattgcgtgcaccacaaataatagcgaagcattgcagattttgcttaaaaaaggagctaagccatgtaaatcaaataaatggggatgtttccctattcaccaagctgcattttcaggttccaaagaatgcatggaaataatactaaggtttggtgaagagcatgggtacagtagacagttgcacattaactttatgaataatgggaaagccacccctctccacctggctgtgcaaaatggtgacttggaaatgatcaaaatgtgcctggacaatggtgcacaaatagacccagtggagaagggaaggtgcacagccattcattttgctgccacccagggagccactgagattgttaaactgatgatatcgtcctattctggtagcgtggatattgttaacacaaccgatggatgtcatgagaccatgcttcacagagcttcattgtttgatcaccatgagctagcagactatttaatttcagtgggagcagatattaataagatcgattctgaaggacgctctccacttatattagcaactgcttctgcatcttggaatattgtaaatttgctactctctaaaggtgcccaagtagacataaaagataattttggacgtaattttctgcatttaactgtacagcaaccttatggattaaaaaatctgcgacctgaatttatgcagatgcaacagatcaaagagctggtaatggatgaagacaacgatgggtgtactcctctacattatgcatgtagacaggggggccctggttctgtaaataacctacttggctttaatgtgtccattcattccaaaagcaaagataagaaatcacctctgcattttgcagccagttatgggcgtatcaatacctgtcagaggctcctacaagacataagtgatacgaggcttctgaatgaaggtgaccttcatggaatgactcctctccatctggcagcaaagaatggacatgataaagtagttcagcttcttctgaaaaaaggtgcattgtttctcagtgaccacaatggctggacagctttgcatcatgcgtccatgggcgggtacactcagaccatgaaggtcattcttgatactaatttgaagtgcacagatcgcctggatgaagacgggaacactgcacttcactttgctgcaagggaaggccacgccaaagccgttgcgcttcttctgagccacaatgctgacatagtcctgaacaagcagcaggcctcctttttgcaccttgcacttcacaataagaggaaggaggttgttcttacgatcatcaggagcaaaagatgggatgaatgtcttaagattttcagtcataattctccaggcaataaatgtccaattacagaaatgatagaatacctccctgaatgcatgaaggtacttttagatttctgcatgttgcattccacagaagacaagtcctgccgagactattatatcgagtataatttcaaatatcttcaatgtccattagaattcaccaaaaaaacacctacacaggatgttatatatgaaccgcttacagccctcaacgcaatggtacaaaataaccgcatagagcttctcaatcatcctgtgtgtaaagaatatttactcatgaaatggttggcttatggatttagagctcatatgatgaatttaggatcttactgtcttggtctcatacctatgaccattctcgttgtcaatataaaaccaggaatggctttcaactcaactggcatcatcaatgaaactagtgatcattcagaaatactagataccacgaattcatatctaataaaaacttgtatgattttagtgtttttatcaagtatatttgggtattgcaaagaagcggggcaaattttccaacagaaaaggaattattttatggatataagcaatgttcttgaatggattatctacacgacgggcatcatttttgtgctgcccttgtttgttgaaataccagctcatctgcagtggcaatgtggagcaattgctgtttacttctattggatgaatttcttattgtatcttcaaagatttgaaaattgtggaatttttattgttatgttggaggtaattttgaaaactttgttgaggtctacagttgtatttatcttccttcttctggcttttggactcagcttttacatcctcctgaatttacaggatcccttcagctctccattgctttctataatccagaccttcagcatgatgctaggagatatcaattatcgagagtccttcctagaaccatatctgagaaatgaattggcacatccagttctgtcctttgcacaacttgtttccttcacaatatttgtcccaattgtcctcatgaatttacttattggtttggcagttggcgacattgctgaggtccagaaacatgcatcattgaagaggatagctatgcaggtggaacttcataccagcttagagaagaagctgccactttggtttctacgcaaagtggatcagaaatccaccatcgtgtatcccaacaaacccagatctggtgggatgttattccatatattctgttttttattttgcactggggaaataagacaagaaataccaaatgctgataaatctttagaaatggaaatattaaagcagaaataccggctgaaggatcttacttttctcctggaaaaacagcatgagctcattaaactgatcattcagaagatggagatcatctctgagacagaggatgatgatagccattgttcttttcaagacaggtttaagaaagagcagatggaacaaaggaatagcagatggaatactgtgttgagagcagtcaaggcaaaaacacaccatcttgagccttag